European Patent Specification EP 3 448 310 B1, published July 31, 2024. Title: COMPOSITIONS AND METHODS FOR GRAFTS MODIFIED WITH A NON-THROMBOGENIC AND PRO-MIGRATORY CELL-DERIVED EXTRACELLULAR MATRIX. Applicant: Yale University Kyriakides, Themis Kristofik, Nina. The sequence listing filed with the application follows.

SEQUENCE LISTING (14 sequences)

SEQ ID NO: 1 - DNA, 23 bp, Artificial Sequence
  Primer
tgactggaagagcggagagtact

SEQ ID NO: 2 - DNA, 19 bp, Artificial Sequence
  Primer
ccttgatggcgtccaggtt

SEQ ID NO: 3 - DNA, 23 bp, Artificial Sequence
  Primer
ctgtaacatggaaactggggaaa

SEQ ID NO: 4 - DNA, 23 bp, Artificial Sequence
  Primer
ccatagctgaactgaaaaccacc

SEQ ID NO: 5 - DNA, 20 bp, Artificial Sequence
  Primer
aacaacgtctgcaacttcgc

SEQ ID NO: 6 - DNA, 20 bp, Artificial Sequence
  Primer
cttcacaaaccgcacacctg

SEQ ID NO: 7 - DNA, 20 bp, Artificial Sequence
  Primer
cttcgccgctactcctgttc

SEQ ID NO: 8 - DNA, 22 bp, Artificial Sequence
  Primer
ccctgagggcaaattgtgaaaa

SEQ ID NO: 9 - DNA, 19 bp, Artificial Sequence
  Primer
ctgctgctacaagcctgct

SEQ ID NO: 10 - DNA, 21 bp, Artificial Sequence
  Primer
ccccataaggtttcagcctca

SEQ ID NO: 11 - DNA, 20 bp, Artificial Sequence
  Primer
gagaggagcactaccccaga

SEQ ID NO: 12 - DNA, 20 bp, Artificial Sequence
  Primer
gcccggattaaggttggtga

SEQ ID NO: 13 - DNA, 20 bp, Artificial Sequence
  Primer
aatgtgggtgtcagctggat

SEQ ID NO: 14 - DNA, 20 bp, Artificial Sequence
  Primer
ctagcaaggttgtgtcgggt